European Patent Application EP 4 509 174 A2, published February 19, 2025. Title: COMPOSITIONS AND METHODS FOR PROMOTING SKIN HEALTH. Applicant: THE REGENTS OF THE UNIVERSITY OF CALIFORNIA. Application EP 17748282.5, filed February 3, 2017. The sequence listing filed with the application follows.

SEQUENCE LISTING (4 sequences)

SEQ ID NO: 1 - DNA, 20 bp, Artificial Sequence
  misc_feature 1..20: note = Synthetic primer
  source 1..20: mol_type = other DNA
gcgcgaggcagacgtgatcc

SEQ ID NO: 2 - DNA, 20 bp, Artificial Sequence
  misc_feature 1..20: note = Synthetic primer
  source 1..20: mol_type = other DNA
gacaccggacctctcccgca

SEQ ID NO: 3 - DNA, 19 bp, Artificial Sequence
  misc_feature 1..19: note = Synthetic primer
  source 1..19: mol_type = other DNA
ctggcacgagaaggaacaa

SEQ ID NO: 4 - DNA, 22 bp, Artificial Sequence
  misc_feature 1..22: note = Synthetic primer
  source 1..22: mol_type = other DNA
gaatcgagcagaactaggtcac